European Patent Application EP 4 480 958 A1, published December 25, 2024. Title: PEPTIDE HAVING ANTIBACTERIAL, ANTIINFLAMMATION OR TISSUE REGENERATION AND USES THEREOF. Applicant: NIBEC Co., Ltd. The sequence listing filed with the application follows.

SEQUENCE LISTING (1 sequence)

SEQ ID NO: 1 - protein, 15 aa, synthetic construct
  REGION 1..15: note = PEPTIDE HAVING ANTIBACTERIAL, ANTIINFLAMMATION OR TISSUE REGENERATION
GKCSTRGRKSSRRKK